European Patent Specification EP 3 479 819 B1, published January 24, 2024. Title: Stable Liquid Pharmaceutical Preparation. Applicant: CELLTRION INC. Application EP 17820536.5. The sequence listing filed with the application follows.

SEQUENCE LISTING (10 sequences)

SEQ ID NO: 1 - protein, 6 aa, Artificial Sequence
  Antibody
QFVGSS

SEQ ID NO: 2 - protein, 3 aa, Artificial Sequence
  Antibody
YAS

SEQ ID NO: 3 - protein, 9 aa, Artificial Sequence
  Antibody
QQSHSWPFT

SEQ ID NO: 4 - protein, 8 aa, Artificial Sequence
  Antibody
GFIFSNHW

SEQ ID NO: 5 - protein, 10 aa, Artificial Sequence
  Antibody
IRSKSINSAT

SEQ ID NO: 6 - protein, 11 aa, Artificial Sequence
  Antibody
SRNYYGSTYDY

SEQ ID NO: 7 - protein, 107 aa, Artificial Sequence
  Antibody
DILLTQSPAILSVSPGERVSFSCRASQFVGSSIHWYQQRTNGSPRLLIKYASESMSGIPSRFSGSGSGTDFTLSINTVESEDIADYYCQQSHSWPFTFGSGTNLEVK

SEQ ID NO: 8 - protein, 119 aa, Artificial Sequence
  Antibody
EVKLEESGGGLVQPGGSMKLSCVASGFIFSNHWMNWVRQSPEKGLEWVAEIRSKSINSATHYAESVKGRFTISRDDSKSAVYLQMTDLRTEDTGVYYCSRNYYGSTYDYWGQGTTLTVS

SEQ ID NO: 9 - protein, 236 aa, Artificial Sequence
  Antibody
MDFQVQIISFLLISASVIMSRGDILLTQSPAILSVSPGERVSFSCRASQFVGSSIHWYQQRTNGSPRLLIKYASESMSGIPSRFSGSGSGTDFTLSINTVESEDIADYYCQQSHSWPFTFGSGTNLEVKRTVAAPSVFIFPPSDEQLKSGTASVVCLLNNFYPREAKVQWKVDNALQSGNSQESVTEQDSKDSTYSLSSTLTLSKADYEKHKVYACEVTHQGLSSPVTKSFNRGEC

SEQ ID NO: 10 - protein, 469 aa, Artificial Sequence
  Antibody
MGWSLILLFLVAVATRVLSEVKLEESGGGLVQPGGSMKLSCVASGFIFSNHWMNWVRQSPEKGLEWVAEIRSKSINSATHYAESVKGRFTISRDDSKSAVYLQMTDLRTEDTGVYYCSRNYYGSTYDYWGQGTTLTVSSASTKGPSVFPLAPSSKSTSGGTAALGCLVKDYFPEPVTVSWNSGALTSGVHTFPAVLQSSGLYSLSSVVTVPSSSLGTQTYICNVNHKPSNTKVDKKVEPKSCDKTHTCPPCPAPELLGGPSVFLFPPKPKDTLMISRTPEVTCVVVDVSHEDPEVKFNWYVDGVEVHNAKTKPREEQYNSTYRVVSVLTVLHQDWLNGKEYKCKVSNKALPAPIEKTISKAKGQPREPQVYTLPPSRDELTKNQVSLTCLVKGFYPSDIAVEWESNGQPENNYKTTPPVLDSDGSFFLYSKLTVDKSRWQQGNVFSCSVMHEALHNHYTQKSLSLSPGK